European Patent Application EP 4 234 683 A1, published August 30, 2023. Title: Modeling atopic dermatitis with human pluripotent stem cell-derived skin organoids. Applicant: Kangstem Biotech CO., LTD. The sequence listing filed with the application follows.

SEQUENCE LISTING (8 sequences)

SEQ ID NO: 1 - DNA, 20 bp, Artificial Sequence
  COL2A_F
catgagggcgcggtagagac

SEQ ID NO: 2 - DNA, 20 bp, Artificial Sequence
  COL2A_R
tccctttggtcctggttgcc

SEQ ID NO: 3 - DNA, 21 bp, Artificial Sequence
  ACAN_F
cttctccggaatggaaacgtg

SEQ ID NO: 4 - DNA, 25 bp, Artificial Sequence
  ACAN_R
acatacctcctggtctatgttacag

SEQ ID NO: 5 - DNA, 20 bp, Artificial Sequence
  SOX9_F
gaagctcgcggaccagtacc

SEQ ID NO: 6 - DNA, 20 bp, Artificial Sequence
  SOX9_R
ctgcccgttcttcaccgact

SEQ ID NO: 7 - DNA, 20 bp, Artificial Sequence
  GAPDH_F
gtcagtggtggacctgacct

SEQ ID NO: 8 - DNA, 20 bp, Artificial Sequence
  GAPDH_R
tgctgtagccaaattcgttg